European Patent Application EP 4 678 754 A2, published January 14, 2026. Title: A MODIFIED MGLUR6 PROMOTER AND METHODS OF USE. Applicant: Wayne State University. Application EP. The sequence listing filed with the application follows.

SEQUENCE LISTING (34 sequences)

SEQ ID NO: 1 - DNA, 202 bp, Mus musculus
  source 1..202: mol_type = genomic DNA
gatctccagatggctaaacttttaaatcatgaatgaagtagatattaccaaattgctttttcagcatccatttagataatcatgttttttgcctttaatctgttaatgtagtgaattacagaaatacatttcctaaatcattacatcccccaaatcgttaatctgctaaagtacatctctggctcaaacaagactggttgtg

SEQ ID NO: 2 - DNA, 198 bp, Homo sapiens
  source 1..198: mol_type = genomic DNA
gatccttagattatgaaacatttacaattatgaatgaatattagatgttatcaaatgctttttctgcatccatttagataatcatgtttttcctttaatctgttaatgcggtgaattacattaatagatttcctaagtcattaatctgctaaagtgcatttctgggacaaaccagacttggttatgacattgtatgta

SEQ ID NO: 3 - DNA, 1095 bp, Mus musculus
  source 1..1095: mol_type = genomic DNA
taaccatgcacgctcgcacacgatagataatacatacaccaatatctgaaaagagaaaaggttctagtggtcaggacagagaatgaaaacggcaggaaggcaagaaagtttgagaacgtagggggtggggtagggagacactacgagtggaataagccacgtttggagaacgtctaggcagatacagaaatgcagaacacagagagaccgagaccagagcagcgtcagaccggctgcaaggctcttgttaggggctttagaaacacctgtgtgctctcccggaagcctggtgcagtcagagaggaagcttgcttcccagacagagatgacacagtttcacaacctgtcagaccaccttgcaggagagactgaaccccagcaaccagaaccacttggctatgcatgtccttttctgtttaaacctaagtctctgaagaccgaccaggggagtccctggacttctttgttcctcttctcggggtggcgggactgattgtgtaaatctcttatctccaactttcactcttatctgtctctttaatcggcatattgaggatgagtggccaagcttattggtgttgctgggtcagacaatttaaaggcagtctaggggagaagcagacccagggagtcagagaggcagagagagaagagagcccttcctccactctcaagctctggagggggtctctgccctcaccctcatccctccccagaatccttaaatcctctagactgtagctctgattttacagctgtcacagactcgtcctactagccagaggttggctcaggtaagcaccactggggaggtagcctagggtgcgctggggtgggtccagaggaagagctgcccagaactgtgggggaaggagcgggaccgaccatcaacagggggacttttcagggagaatgagagcaatcctctggaggcctgggagaggctgctgagttgctggtgcgcgagtcaccaacttttcctgcgctctcggtgtccggccagaatcccgaagtggcagctgagcacggggtggcagcttcgtccgccggctctcaaggcgtcccggtaacttcctttcccgcagtccaggagca

SEQ ID NO: 4 - DNA, 1784 bp, Homo sapiens
  source 1..1784: mol_type = genomic DNA
caagcaggaggctgctgtgtgctgggagctgtcaggctcgtcctgaacagggaagggcccatccacctcccaaacccagtttatgcagtccttcgcaatgtcaggctcagggcctggcaccagccaagctccccacccttcccactgttaaaatggataggagcagggctaggcccagcctgttgactctgggcttccaccaggagaagtggttctggcagtagaaactatcggggcctgggagaggcgggggaagagagaaaggtggcatgtttcttgcttgctccctctaccagccttgtccaaatccccgcagccaccctaatccagcctgtctaatggagcccaagccggctcaggccctcggacgaggagcctgctaatccctgtggctaggagctcaccacctgtctccaggacgccctttgctctcttggcatcagagagccaaatcctgggcctcggatggggggatgataaaagcatcttttggccaagccccctcaccttggcctccacgatgagatggggagttaggtgcagagagcgttggcacagtgagcaccgcagctcgagtggctgcctcagacccagagcccgaggagactttatacggagccagaacgaccccgcggggttccatcctcccaagcaataggcgggagtgggagctgcgaggaaagccggcccctcccctccctccatccaaggcagtgtgggctgtttgtttcatgccattctgggtgtgaatcctgatgcccacacatgccagctgcatgcacttgggcaactcaactcactcctcgagggctgtttctcgactgcagggtgttgtaagttcgctaatactaaaggcttctccctcctggccccttcctgcccctcgctcttcctcctcttccttaggccctcccagctcaggcagcccctgccccctgcagggttctgcaaggagaaagctggggaataccttaggcaactgcagtcaggagcactggtggccaggacagagacagagagacagaaaaggggtcagggacagagagagataaccgcagggagagacaggaagggacagagacagaaaagatttccaagaagaggacagaggcagaaagccagggacagagactgagaaacagagacctagaggcagaagaagactgagatagagatggacagagattgtgtcagacacagccccagagacagccagacagtctgagtcagacgcaaaccaaagacaagaaaacaggaaaacagacccagagattgggagagggaggggaaggagatgcggggagagccagcaccgccaccccccacactcaggaggggtctccaccctcggagcggtctctcatccctccctagaatccttaaatcctctctcgctcagggcctcggccgcatctgtcacagacttgtcctgaaccgacagcggctggcgcaggtgactggcttggggcgggagcctgggtgtgcgctggggatggaccccgaggaagaggggccaagctgtcgggaagcggcagggctggaggggtggaggcagtggtcgggcgggaccccgggcgacagggttcggcgcttgtaagagcgagacggaggcccgggcaggccggctgagctaactccccagagccgaagtggaaggcgcgccccgagcgccttctccccaggaccccggtgtccctccccgcgccccgagcccgcgctctccttcccccgccctcagagcgctccccgcccctctgtctccccgcagcccgctagacgagccg

SEQ ID NO: 5 - DNA, 500 bp, Mus musculus
  source 1..500: mol_type = genomic DNA
ttaaaggcagtctaggggagaagcagacccagggagtcagagaggcagagagagaagagagcccttcctccactctcaagctctggagggggtctctgccctcaccctcatccctccccagaatccttaaatcctctagactgtagctctgattttacagctgtcacagactcgtcctactagccagaggttggctcaggtaagcaccactggggaggtagcctagggtgcgctggggtgggtccagaggaagagctgcccagaactgtgggggaaggagcgggaccgaccatcaacagggggacttttcagggagaatgagagcaatcctctggaggcctgggagaggctgctgagttgctggtgcgcgagtcaccaacttttcctgcgctctcggtgtccggccagaatcccgaagtggcagctgagcacggggtggcagcttcgtccgccggctctcaaggcgtcccggtaacttcctttcccgcagtccaggagca

SEQ ID NO: 6 - DNA, 547 bp, Homo sapiens
  source 1..547: mol_type = genomic DNA
ccaaagacaagaaaacaggaaaacagacccagagattgggagagggaggggaaggagatgcggggagagccagcaccgccaccccccacactcaggaggggtctccaccctcggagcggtctctcatccctccctagaatccttaaatcctctctcgctcagggcctcggccgcatctgtcacagacttgtcctgaaccgacagcggctggcgcaggtgactggcttggggcgggagcctgggtgtgcgctggggatggaccccgaggaagaggggccaagctgtcgggaagcggcagggctggaggggtggaggcagtggtcgggcgggaccccgggcgacagggttcggcgcttgtaagagcgagacggaggcccgggcaggccggctgagctaactccccagagccgaagtggaaggcgcgccccgagcgccttctccccaggaccccggtgtccctccccgcgccccgagcccgcgctctccttcccccgccctcagagcgctccccgcccctctgtctccccgcagcccgctagacgagccg

SEQ ID NO: 7 - DNA, 690 bp, Mus musculus
  source 1..690: mol_type = genomic DNA
ggtgagtcccccaccccactcatcctccctgatgcttcctgtgtgggatgctcatttccacatttgtctcggagtcccacatgctgagtaactctgagatttgctttaaaatgccatgcaggtaatttaaatgggaaggtctgatccaagtgatgaagtgcagccttgatagcatgcttcctccgccctcccacaggcttccatcttttgtggggtgcccacctccacaccttttcttttagctagagtggtcaagtggacaagctggtcattagcaatcaaggcgtttcagatctggaagtgggtggtgccattatggatcagtgagccctgtattttttgtgcctctgcacaaggtgggtagtgaagccctgtccattacataaccatggcatcccctagccatgacataaagggcagtgaaaaattctttaaggatgccagagctgctttttccatttgtgtgtatgcgtgcaggtgtgtgttgtacatgacacaagtgtatgtgtgtgcatgtggaggcctgaggttgatttcaggaatcatcctcaattctttttctaccttattcactgaggcagggtctgtggagagatcaccgatatggctactgtgggattcccctgtctctgccttcagagccactcctggatacacagtacacctggctcagatggtcaccaccctcct

SEQ ID NO: 8 - DNA, 807 bp, Homo sapiens
  source 1..807: mol_type = genomic DNA
tcccccaccccacacgtctccccagcaccccctcttggggatgctcattttctgcatctgtgtaattggtgccataatccagatcccttctcagatccccagatcctatgagtccgatcatctgtggacgcgtccctccaagcagcgcttgactgggatggcgtgcgaggaaagcacgctgacggggaggaattgttgggtttttggttttgtttcttaatttagtgcctgtatttctagaaaccaaggatacggaatataccatcctggtgatcagagtgatgaggcaggaacagatggctcactttacaataggattgctcattttccccaagttgatgacatccttcagggctattttatgaaacacattagggggatatataccatcacgcctggtgcaggtggcagcctggactgagagtagttttagcgataaaggcatctcatcacaagacaggaggtctgagagttggtgactttaggcatggggcagtgagtgtgtggttgccttgggtcttcctgcatagtcacaagatggctgctgaggctccacccattacatcttcacagcagcatcctaacaggaaagagaggctctgagtttgcatcagcatgtaagtgcccaccaatcagaacttggtcacctggccacgcctagctcacctggctcacctggccacgcctaactcacctggccactcctagctcacctggccatgcctagttcacctggccactcctagctcacctggccactcctagctgaaagtgagcaagtggcagaaacacaccctcccccttctt

SEQ ID NO: 9 - DNA, 807 bp, Mus musculus
  source 1..807: mol_type = genomic DNA
actccaggccatgagcaactcctcacatctccctaagcccttcctgtcgccctctggagtcttttgttctgggaatgagacaggcttgactggctgaaggttctccgggcctggcctgggaaacacaggaaaacacgactatttttattgttcattgtgggagagagaactggtaggcaaacccaagagcagaaaatgtaccgtgagggacactgccccagtaaaccctgaaacctacattatcctaagccagccaaggttcttttccagcctgggaagttgagcgtgacattggtggctgaatttgtagacagaatggcttctgagtgcccctgacattccccaaaaggaggctctctgcattaatccatttgtctttattataataaaatatccaagtcagggcgttttttaaggaaaagacttatttttaacatcaactcttggaggtgaaagttcaggcagcgtgacaccagctctgctgaggacctagcttgcatcacattttgacaaatgttatggaaagagggagtagagaaggaaagagtgcatggagagaaggaacatcagaaagaagagggacagggttcactctttgatagctattcaccttcacagaattacctcacccttccagaggtcaagagcaacatccccagtgacccaataaccttgcactaagccacacctcttttttattttttatgagacagggcctcactctgtatccctgaacttgctatgtggaccaagctgtcctcttgagtgctgggattaaaggcattcagtatcagggctggtttataa

SEQ ID NO: 10 - DNA, 673 bp, Homo sapiens
  source 1..673: mol_type = genomic DNA
gggacagtggcacaatcaccgggcccctggggctctccctgagggtcccacccctcctcttgcacatcgccaccttacacactctccctgcctccctttcccctgctccccgcaccccccaccttccctgctgctgcctctgagtctggtgcccaggctcagaagcagcctggtctggggagatgccacaagcccagactgaatagcgcacagaacatgtgtctgtgtttacagctcctgggggtgcggggagggacctgtgggcagaacctagtgcagaaaatgagctgtgagggaaggagcccagggtccatacagaggctgcggaccccagcccgagacccaccggcccgagttcatctccagcctaggaggctgggtgtgacgctggtggaggcatgtggggaggggctggcttcgaactggattttcccccaaggagtccctctgaaccccctgaacagtgggttacagtgggcagagcaagtgggcaggcctagggtcagaggaaagcccagggaaggtgccctaaatgcccccggccccgtttttcctgagaaacaaggatctggtgagtgattatagagcaggggagatggatagagtgggaagggatgggggccgagctggaggaggctcccaggccctccctcaccccagccctgctcctacc

SEQ ID NO: 11 - protein, 712 aa, Chlamydomonas reinhardtii
MSRRPWLLALALAVALAAGSAGASTGSDATVPVATQDGPDYVFHRAHERMLFQTSYTLENNGSVICIPNNGQCFCLAWLKSNGTNAEKLAANILQWITFALSALCLMFYGYQTWKSTCGWEEIYVATIEMIKFIIEYFHEFDEPAVIYSSNGNKTVWLRYAEWLLTCPVILIHLSNLTGLANDYNKRTMGLLVSDIGTIVWGTTAALSKGYVRVIFFLMGLCYGIYTFFNAAKVYIEAYHTVPKGICRDLVRYLAWLYFCSWAMFPVLFLLGPEGFGHINQFNSAIAHAILDLASKNAWSMMGHFLRVKIHEHILLYGDIRKKQKVNVAGQEMEVETMVHEEDDETQKVPTAKYANRDSFIIMRDRLKEKGFETRASLDGDPNGDAEANAAAGGKPGMEMGKMTGMGMGMGAGMGMATIDSGRVILAVPDISMVDFFREQFARLPVPYELVPALGAENTLQLVQQAQSLGGCDFVLMHPEFLRDRSPTGLLPRLKMGGQRAAAFGWAAIGPMRDLIEGSGVDGWLEGPSFGAGINQQALVALINRMQQAKKMGMMGGMGMGMGGGMGMGMGMGMGMAPSMNAGMTGGMGGASMGGAVMGMGMGMQPMQQAMPAMSPMMTQQPSMMSQPSAMSAGGAMQAMGGVMPSPAPGGRVGTNPLFGSAPSPLSSQPGISPGMATPPAATAAPAAGGSEAEMLQQLMSEINRLKNELGE

SEQ ID NO: 12 - protein, 737 aa, Chlamydomonas reinhardtii
MDYGGALSAVGRELLFVTNPVVVNGSVLVPEDQCYCAGWIESRGTNGAQTASNVLQWLAAGFSILLLMFYAYQTWKSTCGWEEIYVCAIEMVKVILEFFFEFKNPSMLYLATGHRVQWLRYAEWLLTCPVILIHLSNLTGLSNDYSRRTMGLLVSDIGTIVWGATSAMATGYVKVIFFCLGLCYGANTFFHAAKAYIEGYHTVPKGRCRQVVTGMAWLFFVSWGMFPILFILGPEGFGVLSVYGSTVGHTIIDLMSKNCWGLLGHYLRVLIHEHILIHGDIRKTTKLNIGGTEIEVETLVEDEAEAGAVNKGTGKYASRESFLVMRDKMKEKGIDVRASLDNSKEVEQEQAARAAMMMMNGNGMGMGMGMNGMNGMGGMNGMAGGAKPGLELTPQLQPGRVILAVPDISMVDFFREQFAQLSVTYELVPALGADNTLALVTQAQNLGGVDFVLIHPEFLRDRSSTSILSRLRGAGQRVAAFGWAQLGPMRDLIESANLDGWLEGPSFGQGILPAHIVALVAKMQQMRKMQQMQQIGMMTGGMNGMGGGMGGGMNGMGGGNGMNNMGNGMGGGMGNGMGGNGMNGMGGGNGMNNMGGNGMAGNGMGGGMGGNGMGGSMNGMSSGVVANVTPSAAGGMGGMMNGGMAAPQSPGMNGGRLGTNPLFNAAPSPLSSQLGAEAGMGSMGGMGGMSGMGGMGGMGGMGGAGAATTQAAGGNAEAEMLQNLMNEINRLKRELGE

SEQ ID NO: 13 - protein, 315 aa, Chlamydomonas reinhardtii
MDYGGALSAVGRELLFVTNPVVVNGSVLVPEDQCYCAGWIESRGTNGAQTASNVLQWLAAGFSILLLMFYAYQTWKSTCGWEEIYVCAIEMVKVILEFFFEFKNPSMLYLATGHRVQWLRYAEWLLTCPVILIHLSNLTGLSNDYSRRTMGLLVSDIGTIVWGATSAMATGYVKVIFFCLGLCYGANTFFHAAKAYIEGYHTVPKGRCRQVVTGMAWLFFVSWGMFPILFILGPEGFGVLSVYGSTVGHTIIDLMSKNCWGLLGHYLRVLIHEHILIHGDIRKTTKLNIGGTEIEVETLVEDEAEAGAVNKGTGK

SEQ ID NO: 14 - protein, 837 aa, synthetic construct
MDYPVARSLIVRYPTDLGNGTVCMPRGQCYCEGWLRSRGTSIEKTIAITLQWVVFALSVACLGWYAYQAWRATCGWEEVYVALIEMMKSIIEAFHEFDSPATLWLSSGNGVVWMRYGEWLLTCPVLLIHLSNLTGLKDDYSKRTMGLLVSDVGCIVWGATSAMCTGWTKILFFLISLSYGMYTYFHAAKVYIEAFHTVPKGICRELVRVMAWTFFVAWGMFPVLFLLGTEGFGHISPYGSAIGHSILDLIAKNMWGVLGNYLRVKIHEHILLYGDIRKKQKITIAGQEMEVETLVAEEEDDTVKQSTAKYASRDSFITMRNRMREKGLEVRASLDAGGGDSGMEAGGGGAAHAQPHMAKPGTELGKTMSASFTNGAATSLEPGRVILAVPDISMVDFFREQFAQLPVPYEVVPALGAENTVQLVQQAAMLGGCDFVLMHPEFLRDRGPTGLLPQVKMMGQRTAAFGWSQMGPMRDLIESSGVGAWLEGPSFGSGISQAALQQLVVKMQQAKRMAAMGSMMGGGMGNGMGMGMGMGMGMGMGNGMGNGMGMGNGMGNGMGMGNGMGNGMGMGNGMGMGNGMGMGNGMGMGNGMGNGMGNGMGMGNGMGNGMGNGMGNGMGNGMGNGMGMGNGMGMGNGMGNGMGNGMGNGMGNGMGMMTPGAMGMGMGGMGNLAAAAGNAMYGGGGGGGGSTMGSGNAAMMTGLVMGGGNGVGAGPGGVVANLGSSALQPQSQMMGGGNVVGMSSPQLQLQQSSSMPLGGLAPNRIGNNPLFGAAPSPLHSQPGASPTGLSSPQLGMGAMLPAGTSVGAGGGSVGPTETDMLQQLMTEINRLKDELGE

SEQ ID NO: 15 - protein, 747 aa, synthetic construct
MDHPVARSLIGSSYTNLNNGSIVIPSDACFCMKWLKSKGSPVALKMANALQWAAFALSVIILIYYAYATWRTTCGWEEVYVCCVELTKVVIEFFHEFDEPGMLYLANGNRVLWLRYGEWLLTCPVILIHLSNLTGLKDDYNKRTMRLLVSDVGTIVWGATAAMSTGYIKVIFFLLGCMYGANTFFHAAKVYIESYHTVPKGLCRQLVRAMAWLFFVSWGMFPVLFLLGPEGFGHLSVYGSTIGHTIIDLLSKNCWGLLGHFLRLKIHEHILLYGDIRKVQKIRVAGEELEVETLMTEEAPDTVKKSTAQYANRESFLTMRDKLKEKGFEVRASLDNSGIDAVINHNNNYNNALANAAAAVGKPGMELSKLDHVAANAAGMGGIADHVATTSGAISPGRVILAVPDISMVDYFREQFAQLPVQYEVVPALGADNAVQLVVQAAGLGGCDFVLLHPEFLRDKSSTSLPARLRSIGQRVAAFGWSPVGPVRDLIESAGLDGWLEGPSFGLGISLPNLASLVLRMQHARKMAAMLGGMGGMLGSNLMSGSGGVGLMGAGSPGGGGGAMGVGMTGMGMVGTNAMGRGAVGNSVANASMGGGSAGMGMGMMGMVGAGVGGQQQMGANGMGPTSFQLGSNPLYNTAPSPLSSQPGGDASAAAAAAAAAAATGAASNSMNAMQAGGSVRNSGILAGGLGSMMGPPGAPAAPTAAATAAPAVTMGAPGGGGAAASEAEMLQQLMAEINRLKSELGE

SEQ ID NO: 16 - protein, 291 aa, Natronomonas pharaonis
MTETLPPVTESAVALQAEVTQRELFEFVLNDPLLASSLYINIALAGLSILLFVFMTRGLDDPRAKLIAVSTILVPVVSIASYTGLASGLTISVLEMPAGHFAEGSSVMLGGEEVDGVVTMWGRYLTWALSTPMILLALGLLAGSNATKLFTAITFDIAMCVTGLAAALTTSSHLMRWFWYAISCACFLVVLYILLVEWAQDAKAAGTADMFNTLKLLTVVMWLGYPIVWALGVEGIAVLPVGVTSWGYSFLDIVAKYIFAFLLLNYLTSNESVVSGSILDVPSASGTPADD

SEQ ID NO: 17 - protein, 521 aa, Mus musculus
MDSPSGPRVLSSLTQDPSFTTSPALQGIWNGTQNVSVRAQLLSVSPTTSAHQAAAWVPFPTVDVPDHAHYTLGTVILLVGLTGMLGNLTVIYTFCRNRGLRTPANMFIINLAVSDFLMSVTQAPVFFASSLYKKWLFGETGCEFYAFCGAVFGITSMITLTAIAMDRYLVITRPLATIGRGSKRRTALVLLGVWLYALAWSLPPFFGWSAYVPEGLLTSCSWDYMTFTPQVRAYTMLLFCFVFFLPLLIIIFCYIFIFRAIRETGRACEGCGESPLRQRRQWQRLQSEWKMAKVALIVILLFVLSWAPYSTVALVAFAGYSHILTPYMSSVPAVIAKASAIHNPIIYAITHPKYRVAIAQHLPCLGVLLGVSGQRSHPSLSYRSTHRSTLSSQSSDLSWISGRKRQESLGSESEVGWTDTETTAAWGAAQQASGQSFCSQNLEDGELKASSSPQVQRSKTPKVPGPSTCRPMKGQGARPSSLRGDQKGRLAVCTGLSECPHPHTSQFPLAFLEDDVTLRHL

SEQ ID NO: 18 - protein, 478 aa, Homo sapiens
MNPPSGPRVLPSPTQEPSCMATPAPPSWWDSSQSSISSLGRLPSISPTAPGTWAAAWVPLPTVDVPDHAHYTLGTVILLVGLTGMLGNLTVIYTFCRSRSLRTPANMFIINLAVSDFLMSFTQAPVFFTSSLYKQWLFGETGCEFYAFCGALFGISSMITLTAIALDRYLVITRPLATFGVASKRRAAFVLLGVWLYALAWSLPPFFGWSAYVPEGLLTSCSWDYMSFTPAVRAYTMLLCCFVFFLPLLIIIYCYIFIFRAIRETGRALQTFGACKGNGESLWQRQRLQSECKMAKIMLLVILLFVLSWAPYSAVALVAFAGYAHVLTPYMSSVPAVIAKASAIHNPIIYAITHPKYRVAIAQHLPCLGVLLGVSRRHSRPYPSYRSTHRSTLTSHTSNLSWISIRRRQESLGSESEVGWTHMEAAAVWGAAQQANGRSLYGQGLEDLEAKAPPRPQGHEAETPGKTKGLIPSQDPRM

SEQ ID NO: 19 - DNA, 514 bp, Homo sapiens
  source 1..514: mol_type = other DNA
gtcgagagatctacgggtggcatccctgtgacccctccccagtgcctctcctggccctggaagttgccactccagtgcccaccagccttgtcctaataaaattaagttgcatcattttgtctgactaggtgtccttctataatattatggggtggaggggggtggtatggagcaaggggcaagttgggaagacaacctgtagggcctgcggggtctattgggaaccaagctggagtgcagtggcacaatcttggctcactgcaatctccgcctcctgggttcaagcgattctcctgcctcagcctcccgagttgttgggattccaggcatgcatgaccaggctcagctaatttttgtttttttggtagagacggggtttcaccatattggccaggctggtctccaactcctaatctcaggtgatctacccaccttggcctcccaaattgctgggattacaggcgtgaaccactgctcccttccctgtccttctgattttgtaggtaaccacgtg

SEQ ID NO: 20 - DNA, 2161 bp, synthetic construct
  misc_feature 1..2161: note = Mutated capsid protein
  source 1..2161: mol_type = other DNA
tcagagagagtgtcctcgagccaatctgaaacaataccatcggcagccatacctgatttaaatcatttattgttcaaagatgcagtcatccaaatccacattgaccagatcgcaggcagtgcaagcgtctggcacctttcccatgatatgatgaatgtagcacagtttctgatacgcctttttgacgacagaaacgggttgagattctgacacgggaaagcactctaaacagtctttctgtccgtgagtgaagcagatatttgaattctgattcattctctcgcattgtctgcagggaaacagcatcagattcatgcccacgtgacgagaacatttgttttggtacctgtctgcgtagttgatcgaagcttccgcgtctgacgtcgatggctgcgcaactgactcgcgcacccgtttgggctcacttatatctgcgtcactgggggcgggtcttttcttggctccaccctttttgacgtagaattcatgctccacctcaaccacgtgatcctttgcccaccggaaaaagtctttgacttcctgcttggtgaccttcccaaagtcatgatccagacggcgggtgagttcaaatttgaacatccggtcttgcaacggctgctggtgttcgaaggtcgttgagttcccgtcaatcacggcgcacatgttggtgttggaggtgacgatcacgggagtcgggtctatctgggccgaggacttgcatttctggtccacgcgcaccttgcttcctccgagaatggctttggccgactccacgaccttggcggtcatcttcccctcctcccaccagatcaccatcttgtcgacacagtcgttgaagggaaagttctcattggtccagtttacgcacccgtagaagggcacagtgtgggctatggcctccgcgatgttggtcttcccggtagttgcaggcccaaacagccagatggtgttcctcttgccgaactttttcgtggcccatcccagaaagacggaagccgcatattggggatcgtacccgtttagttccaaaattttataaatccgattgctggaaatgtcctccacgggctgctggcccaccaggtagtcgggggcggttttagtcaggctcataatctttcccgcattgtccaaggcagccttgatttgggaccgcgagttggaggccgcattgaaggagatgtatgaggcctggtcctcctggatccactgcttctccgaggtaatccccttgtccacgagccacccgaccagctccatgtacctggctgaagtttttgatctgatcaccggcgcatcagaattgggattctgattctctttgttctgctcctgcgtctgcgacacgtgcgtcagatgctgcgccaccaaccgtttacgctccgtgagattcaaacaggcgctgaaacaataggaagggagtggatgtcagtgtgtgctgcccgggggctctgactacaggtctcccccttcgcgcccgatggtgggacggtatgaataatccggaatatttataggtttttttattacaaaactgttacgaaaacagtaaaatacttatttatttgcgagatggttatcattttaattatctccatgatagatctctatcactgatagggagtacttaccttaaatactgttccatattagtccacgcccactggagctcaggctgggttttggggagcaagtaattggggatgtagcactcatccaccaccttgttcccgcctccggcgccatttctggtctttgtgaccgcgaaccagtttggcaaagtcggctcgatcccgcggtaaattctctgaatcagtttttcgcgaatctgactcaggaaacgtcccaaaaccatggatttcaccccggtggtttccacgagcacgtgcatgtggaagtagctctctcccttctcaaattgcacaaagaaaagggcctccggggccttactcacacggcgccattccgtcagaaagtcgcgctgcagcttctcggccacggtcaggggtgcctgctcaatcagattcagatccatgtcagaatctggcggcaactcccattccttctcggccacccagttcacaaagctgtcagaaatgccgggcagatgctcgtcaaggtcgctggggaccttaatcacaatctcgtaaaaccccggcat

SEQ ID NO: 21 - DNA, 6057 bp, synthetic construct
  misc_feature 1..6057: note = Vector V-032-pFB-AAV-CMV-SV40pA
  source 1..6057: mol_type = other DNA
gacgcgccctgtagcggcgcattaagcgcggcgggtgtggtggttacgcgcagcgtgaccgctacacttgccagcgccctagcgcccgctcctttcgctttcttcccttcctttctcgccacgttcgccggctttccccgtcaagctctaaatcgggggctccctttagggttccgatttagtgctttacggcacctcgaccccaaaaaacttgattagggtgatggttcacgtagtgggccatcgccctgatagacggtttttcgccctttgacgttggagtccacgttctttaatagtggactcttgttccaaactggaacaacactcaaccctatctcggtctattcttttgatttataagggattttgccgatttcggcctattggttaaaaaatgagctgatttaacaaaaatttaacgcgaattttaacaaaatattaacgtttacaatttcaggtggcacttttcggggaaatgtgcgcggaacccctatttgtttatttttctaaatacattcaaatatgtatccgctcatgagacaataaccctgataaatgcttcaataatattgaaaaaggaagagtatgagtattcaacatttccgtgtcgcccttattcccttttttgcggcattttgccttcctgtttttgctcacccagaaacgctggtgaaagtaaaagatgctgaagatcagttgggtgcacgagtgggttacatcgaactggatctcaacagcggtaagatccttgagagttttcgccccgaagaacgttttccaatgatgagcacttttaaagttctgctatgtggcgcggtattatcccgtattgacgccgggcaagagcaactcggtcgccgcatacactattctcagaatgacttggttgagtactcaccagtcacagaaaagcatcttacggatggcatgacagtaagagaattatgcagtgctgccataaccatgagtgataacactgcggccaacttacttctgacaacgatcggaggaccgaaggagctaaccgcttttttgcacaacatgggggatcatgtaactcgccttgatcgttgggaaccggagctgaatgaagccataccaaacgacgagcgtgacaccacgatgcctgtagcaatggcaacaacgttgcgcaaactattaactggcgaactacttactctagcttcccggcaacaattaatagactggatggaggcggataaagttgcaggaccacttctgcgctcggcccttccggctggctggtttattgctgataaatctggagccggtgagcgtgggtctcgcggtatcattgcagcactggggccagatggtaagccctcccgtatcgtagttatctacacgacggggagtcaggcaactatggatgaacgaaatagacagatcgctgagataggtgcctcactgattaagcattggtaactgtcagaccaagtttactcatatatactttagattgatttaaaacttcatttttaatttaaaaggatctaggtgaagatcctttttgataatctcatgaccaaaatcccttaacgtgagttttcgttccactgagcgtcagaccccgtagaaaagatcaaaggatcttcttgagatcctttttttctgcgcgtaatctgctgcttgcaaacaaaaaaaccaccgctaccagcggtggtttgtttgccggatcaagagctaccaactctttttccgaaggtaactggcttcagcagagcgcagataccaaatactgtccttctagtgtagccgtagttaggccaccacttcaagaactctgtagcaccgcctacatacctcgctctgctaatcctgttaccagtggctgctgccagtggcgataagtcgtgtcttaccgggttggactcaagacgatagttaccggataaggcgcagcggtcgggctgaacggggggttcgtgcacacagcccagcttggagcgaacgacctacaccgaactgagatacctacagcgtgagcattgagaaagcgccacgcttcccgaagggagaaaggcggacaggtatccggtaagcggcagggtcggaacaggagagcgcacgagggagcttccagggggaaacgcctggtatctttatagtcctgtcgggtttcgccacctctgacttgagcgtcgatttttgtgatgctcgtcaggggggcggagcctatggaaaaacgccagcaacgcggcctttttacggttcctggccttttgctggccttttgctcacatgttctttcctgcgttatcccctgattctgtggataaccgtattaccgcctttgagtgagctgataccgctcgccgcagccgaacgaccgagcgcagcgagtcagtgagcgaggaagcggaagagcgcctgatgcggtattttctccttacgcatctgtgcggtatttcacaccgcagaccagccgcgtaacctggcaaaatcggttacggttgagtaataaatggatgccctgcgtaagcgggtgtgggcggacaataaagtcttaaactgaacaaaatagatctaaactatgacaataaagtcttaaactagacagaatagttgtaaactgaaatcagtccagttatgctgtgaaaaagcatactggacttttgttatggctaaagcaaactcttcattttctgaagtgcaaattgcccgtcgtattaaagaggggcgtggccaagggcatggtaaagactatattcgcggcgttgtgacaatttaccgaacaactccgcggccgggaagccgatctcggcttgaacgaattgttaggtggcggtacttgggtcgatatcaaagtgcatcacttcttcccgtatgcccaactttgtatagagagccactgcgggatcgtcaccgtaatctgcttgcacgtagatcacataagcaccaagcgcgttggcctcatgcttgaggagattgatgagcgcggtggcaatgccctgcctccggtgctcgccggagactgcgagatcatagatatagatctcactacgcggctgctcaaacctgggcagaacgtaagccgcgagagcgccaacaaccgcttcttggtcgaaggcagcaagcgcgatgaatgtcttactacggagcaagttcccgaggtaatcggagtccggctgatgttgggagtaggtggctacgtctccgaactcacgaccgaaaagatcaagagcagcccgcatggatttgacttggtcagggccgagcctacatgtgcgaatgatgcccatacttgagccacctaactttgttttagggcgactgccctgctgcgtaacatcgttgctgctgcgtaacatcgttgctgctccataacatcaaacatcgacccacggcgtaacgcgcttgctgcttggatgcccgaggcatagactgtacaaaaaaacagtcataacaagccatgaaaaccgccactgcgccgttaccaccgctgcgttcggtcaaggttctggaccagttgcgtgagcgcatacgctacttgcattacagtttacgaaccgaacaggcttatgtcaactgggttcgtgccttcatccgtttccacggtgtgcgtcacccggcaaccttgggcagcagcgaagtcgaggcatttctgtcctggctggcgaacgagcgcaaggtttcggtctccacgcatcgtcaggcattggcggccttgctgttcttctacggcaaggtgctgtgcacggatctgccctggcttcaggagatcggaagacctcggccgtcgcggcgcttgccggtggtgctgaccccggatgaagtggttcgcatcctcggttttctggaaggcgagcatcgtttgttcgcccaggactctagctatagttctagtggttggctacattattgaagcatttatcagggttattgtctcagagcatgcctgcaggcagctgcgcgctcgctcgctcactgaggccgcccgggcgtcgggcgacctttggtcgcccggcctcagtgagcgagcgagcgcgcagagagggagtggccaactccatcactaggggttcctgcggccgcacgcgtgttactagttattaatagtaatcaattacggggtcattagttcatagcccatatatggagttccgcgttacataacttacggtaaatggcccgcctggctgaccgcccaacgacccccgcccattgacgtcaataatgacgtatgttcccatagtaacgccaatagggactttccattgacgtcaatgggtggagtatttacggtaaactgcccacttggcagtacatcaagtgtatcatatgccaagtacgccccctattgacgtcaatgacggtaaatggcccgcctggcattatgcccagtacatgaccttatgggactttcctacttggcagtacatctacgtattagtcatcgctattaccatggtgatgcggttttggcagtacatcaatgggcgtggatagcggtttgactcacggggatttccaagtctccaccccattgacgtcaatgggagtttgttttggcaccaaaatcaacgggactttccaaaatgtcgtaacaactccgccccattgacgcaaatgggcggtaggcgtgtacggtgggaggtctatataagcagagctcgtttagtgaaccgtcagatcgcctggagacgccatccacgctgttttgacctccatagaagacaccgggaccgatccagcctccaaccggttcgaacaggtaagcgcccctaaaatccctttggcacaatgtgtcctgaggggagaggcagcgacctgtagatgggacgggggcactaaccctcagggtttggggttctgaatgtgagtatcgccatgtaagcccagtatttggccaatctcagaaagctcctggctccctggaggatggagagagaaaaacaaacagctcctggagcagggagagtgctggcctcttgctctccggctccctctgttgccctctggtttctccccaggttgaattcgatatcggatccatcgataccgtcgacctcgagggggggcccggtacccaattcgccctatagtgagtcgtattacgcgcgcagcggccgaccatggcccaacttgtttattgcagcttataatggttacaaataaagcaatagcatcacaaatttcacaaataaagcatttttttcactgcattctagttgtggtttgtccaaactcatcaatgtatcttatcatgtctggatctccggaccacgtgcggaccgagcggccgcaggaacccctagtgatggagttggccactccctctctgcgcgctcgctcgctcactgaggccgggcgaccaaaggtcgcccgacgcccgggctttgcccgggcggcctcagtgagcgagcgagcgcgcagctgcctgcaggaagctgtaagcttgtcgagaagtactagaggatcataatcagccataccacatttgtagaggttttacttgctttaaaaaacctcccacacctccccctgaacctgaaacataaaatgaatgcaattgttgttgttaacttgtttattgcagcttataatggttacaaataaagcaatagcatcacaaatttcacaaataaagcatttttttcactgcattctagttgtggtttgtccaaactcatcaatgtatcttatcatgtctggatctgatcactgatatcgcctaggagatccgaaccagataagtgaaatctagttccaaactattttgtcatttttaattttcgtattagcttacgacgctacacccagttcccatctattttgtcactcttccctaaataatccttaaaaactccatttccacccctcccagttcccaactattttgtccgcccacagcggggcatttttcttcctgttatgtttttaatcaaacatcctgccaactccatgtgacaaaccgtcatcttcggctactttttctctgtcacagaatgaaaatttttctgtcatctcttcgttattaatgtttgtaattgactgaatatcaacgcttatttgcagcctgaatggcgaatg

SEQ ID NO: 22 - DNA, 10078 bp, synthetic construct
  misc_feature 1..10078: note = Vector V117-pFB-inCap2-Y444F-inRepOpt-Kan
  source 1..10078: mol_type = other DNA
ttctctgtcacagaatgaaaatttttctgtcatctcttcgttattaatgtttgtaattgactgaatatcaacgcttatttgcagcctgaatggcgaatgggacgcgccctgtagcggcgcattaagcgcggcgggtgtggtggttacgcgcagcgtgaccgctacacttgccagcgccctagcgcccgctcctttcgctttcttcccttcctttctcgccacgttcgccggctttccccgtcaagctctaaatcgggggctccctttagggttccgatttagtgctttacggcacctcgaccccaaaaaacttgattagggtgatggttcacgtagtgggccatcgccctgatagacggtttttcgccctttgacgttggagtccacgttctttaatagtggactcttgttccaaactggaacaacactcaaccctatctcggtctattcttttgatttataagggattttgccgatttcggcctattggttaaaaaatgagctgatttaacaaaaatttaacgcgaattttaacaaaatattaacgtttacaatttcctgatgcggtattttctccttacgcatctgtgcggtatttcacaccgcatatggtgcactctcagtacaatctgctctgatgccgcatagttaagccagccccgacacccgccaacacccgctgacgcgccctgacgggcttgtctgctcccggcatccgcttacagacaagctgtgaccgtctccgggagctgcatgtgtcagaggttttcaccgtcatcaccgaaacgcgcgagacgaaagggcctcgtgatacgcctatttttataggttaatgtcatgataataatggtttcttagacgtcaggtggcacttttcggggaaatgtgcgcggaacccctatttgtttatttttctaaatacattcaaatatgtatccgctcatgagacaataaccctgataaatgcttcaataatattgaaaaaggaagagtatgattgaacaagatggattgcacgcaggttctccggccgcttgggtggagaggctattcggctatgactgggcacaacagacaatcggctgctctgatgccgccgtgttccggctgtcagcgcaggggcgcccggttctttttgtcaagaccgacctgtccggtgccctgaatgaactgcaggacgaggcagcgcggctatcgtggctggccacgacgggcgttccttgcgcagctgtgctcgacgttgtcactgaagcgggaagggactggctgctattgggcgaagtgccggggcaggatctcctgtcatctcaccttgctcctgccgagaaagtatccatcatggctgatgcaatgcggcggctgcatacgcttgatccggctacctgcccattcgaccaccaagcgaaacatcgcatcgagcgagcacgtactcggatggaagccggtcttgtcgatcaggatgatctggacgaagagcatcaggggctcgcgccagccgaactgttcgccaggctcaaggcgcgcatgcccgacggcgaggatctcgtcgtgacccatggcgatgcctgcttgccgaatatcatggtggaaaatggccgcttttctggattcatcgactgtggccggctgggtgtggcggaccgctatcaggacatagcgttggctacccgtgatattgctgaagagcttggcggcgaatgggctgaccgcttcctcgtgctttacggtatcgccgctcccgattcgcagcgcatcgccttctatcgccttcttgacgagttcttctgagtaaccgtcagaccaagtttactcatatatactttagattgatttaaaacttcatttttaatttaaaaggatctaggtgaagatcctttttgataatctcatgaccaaaatcccttaacgtgagttttcgttccactgagcgtcagaccacgtagaaaagatcaaaggatcttcttgagatcctttttttctgcgcgtaatctgctgcttgcaaacaaaaaaaccaccgctaccagcggtggtttgtttgccggatcaagagctaccaactctttttccgaaggtaactggcttcagcagagcgcagataccaaatactgtccttctagtgtagccgtagttaggccaccacttcaagaactctgtagcaccgcctacatacctcgctctgctaatcctgttaccagtggctgctgccagtggcgataagtcgtgtcttaccgggttggactcaagacgatagttaccggataaggcgcagcggtcgggctgaacggggggttcgtgcacacagcccagcttggagcgaacgacctacaccgaactgagatacctacagcgtgagcattgagaaagcgccacgcttcccgaagggagaaaggcggacaggtatccggtaagcggcagggtcggaacaggagagcgcacgagggagcttccagggggaaacgcctggtatctttatagtcctgtcgggtttcgccacctctgacttgagcgtcgatttttgtgatgctcgtcaggggggcggagcctatggaaaaacgccagcaacgcggcctttttacggttcctggccttttgctggccttttgctcacatgttctttcctgcgttatcccctgattctgtggataaccgtattaccgcctttgagtgagctgataccgctcgccgcagccgaacgaccgagcgcagcgagtcagtgagcgaggaagcggaagagcgcctgatgcggtattttctccttacgcatctgtgcggtatttcacaccgcagaccagccgcgtaacctggcaaaatcggttacggttgagtaataaatggatgccctgcgtaagcgggtgtgggcggacaataaagtcttaaactgaacaaaatagatctaaactatgacaataaagtcttaaactagacagaatagttgtaaactgaaatcagtccagttatgctgtgaaaaagcatactggacttttgttatggctaaagcaaactcttcattttctgaagtgcaaattgcccgtcgtattaaagaggggcgtggccaagggcatggtaaagactatattcgcggcgttgtgacaatttaccgaacaactccgcggccgggaagccgatctcggcttgaacgaattgttaggtggcggtacttgggtcgatatcaaagtgcatcacttcttcccgtatgcccaactttgtatagagagccactgcgggatcgtcaccgtaatctgcttgcacgtagatcacataagcaccaagcgcgttggcctcatgcttgaggagattgatgagcgcggtggcaatgccctgcctccggtgctcgccggagactgcgagatcatagatatagatctcactacgcggctgctcaaacctgggcagaacgtaagccgcgagagcgccaacaaccgcttcttggtcgaaggcagcaagcgcgatgaatgtcttactacggagcaagttcccgaggtaatcggagtccggctgatgttgggagtaggtggctacgtctccgaactcacgaccgaaaagatcaagagcagcccgcatggatttgacttggtcagggccgagcctacatgtgcgaatgatgcccatacttgagccacctaactttgttttagggcgactgccctgctgcgtaacatcgttgctgctgcgtaacatcgttgctgctccataacatcaaacatcgacccacggcgtaacgcgcttgctgcttggatgcccgaggcatagactgtacaaaaaaacagtcataacaagccatgaaaaccgccactgcgccgttaccaccgctgcgttcggtcaaggttctggaccagttgcgtgagcgcatacgctacttgcattacagtttacgaaccgaacaggcttatgtcaactgggttcgtgccttcatccgtttccacggtgtgcgtcacccggcaaccttgggcagcagcgaagtcgaggcatttctgtcctggctggcgaacgagcgcaaggtttcggtctccacgcatcgtcaggcattggcggccttgctgttcttctacggcaaggtgctgtgcacggatctgccctggcttcaggagatcggtagacctcggccgtcgcggcgcttgccggtggtgctgaccccggatgaagtggttcgcatcctcggttttctggaaggcgagcatcgtttgttcgcccaggactctagctatagttctagtggttggcctacgtacccgtagtggctatggcagggcttgccgccccgacgttggctgcgagccctgggccttcacccgaacttgggggttggggtggggaaaaggaagaaacgcgggcgtattggtcccaatggggtctcggtggggtatcgacagagtgccagccctgggaccgaaccccgcgtttatgaacaaacgacccaacacccgtgcgttttattctgtctttttattgccgtcatagcgcgggttccttccggtattgtctccttccgtgtttcagttagcctcccccatctcccggtaccgcatgctccttcagagagagtgtcctcgagccaatctgaaacaataccatcggcagccatacctgatttaaatcatttattgttcaaagatgcagtcatccaaatccacattgaccagatcgcaggcagtgcaagcgtctggcacctttcccatgatatgatgaatgtagcacagtttctgatacgcctttttgacgacagaaacgggttgagattctgacacgggaaagcactctaaacagtctttctgtccgtgagtgaagcagatatttgaattctgattcattctctcgcattgtctgcagggaaacagcatcagattcatgcccacgtgacgagaacatttgttttggtacctgtctgcgtagttgatcgaagcttccgcgtctgacgtcgatggctgcgcaactgactcgcgcacccgtttgggctcacttatatctgcgtcactgggggcgggtcttttcttggctccaccctttttgacgtagaattcatgctccacctcaaccacgtgatcctttgcccaccggaaaaagtctttgacttcctgcttggtgaccttcccaaagtcatgatccagacggcgggtgagttcaaatttgaacatccggtcttgcaacggctgctggtgttcgaaggtcgttgagttcccgtcaatcacggcgcacatgttggtgttggaggtgacgatcacgggagtcgggtctatctgggccgaggacttgcatttctggtccacgcgcaccttgcttcctccgagaatggctttggccgactccacgaccttggcggtcatcttcccctcctcccaccagatcaccatcttgtcgacacagtcgttgaagggaaagttctcattggtccagtttacgcacccgtagaagggcacagtgtgggctatggcctccgcgatgttggtcttcccggtagttgcaggcccaaacagccagatggtgttcctcttgccgaactttttcgtggcccatcccagaaagacggaagccgcatattggggatcgtacccgtttagttccaaaattttataaatccgattgctggaaatgtcctccacgggctgctggcccaccaggtagtcgggggcggttttagtcaggctcataatctttcccgcattgtccaaggcagccttgatttgggaccgcgagttggaggccgcattgaaggagatgtatgaggcctggtcctcctggatccactgcttctccgaggtaatccccttgtccacgagccacccgaccagctccatgtacctggctgaagtttttgatctgatcaccggcgcatcagaattgggattctgattctctttgttctgctcctgcgtctgcgacacgtgcgtcagatgctgcgccaccaaccgtttacgctccgtgagattcaaacaggcgctgaaacaataggaagggagtggatgtcagtgtgtgctgcccgggggctctgactacaggtctcccccttcgcgcccgatggtgggacggtatgaataatccggaatatttataggtttttttattacaaaactgttacgaaaacagtaaaatacttatttatttgcgagatggttatcattttaattatctccatgatagatctctatcactgatagggagtacttaccttaaatactgttccatattagtccacgcccactggagctcaggctgggttttggggagcaagtaattggggatgtagcactcatccaccaccttgttcccgcctccggcgccatttctggtctttgtgaccgcgaaccagtttggcaaagtcggctcgatcccgcggtaaattctctgaatcagtttttcgcgaatctgactcaggaaacgtcccaaaaccatggatttcaccccggtggtttccacgagcacgtgcatgtggaagtagctctctcccttctcaaattgcacaaagaaaagggcctccggggccttactcacacggcgccattccgtcagaaagtcgcgctgcagcttctcggccacggtcaggggtgcctgctcaatcagattcagatccatgtcagaatctggcggcaactcccattccttctcggccacccagttcacaaagctgtcagaaatgccgggcagatgctcgtcaaggtcgctggggaccttaatcacaatctcgtaaaaccccggcatggcgggtagggtgatcaagtcttcgtcgagtgattgtaaataaaatgtaatttacagtatagtattttaattaatatacaaatgatttgataataattcttatttaactataatatattgtgttgggttgaattaaaggtccgtagctttcgaatctaggctcaagcagtgatcagatccagacatgataagatacattgatgagtttggacaaaccacaactagaatgcagtgaaaaaaatgctttatttgtgaaatttgtgatgctattgctttatttgtaaccattataagctgcaataaacaagttaacaacaacaattgcattcattttatgtttcaggttcagggggaggtgtgggaggttttttaaagcaagtaaaacctctacaaatgtggtatggctgattatgatcctctagtacttctcgacaagctgtagccatggaaactagataagaaagaaatacgcagagaccaaagttcaactgaaacgaattaaacggtttattgattaacaagcaattacagattacgagtcaggtatctggtgccaatggggcgaggctctgaatacacgccattagtgtccacagtaaagtccacattaacagacttgttgtagttggaagtgtactgaatttcgggattccagcgtttgctgttttccttctgcagctcccactcgatctccacgctgacctgtcccgtggagtactgtgtgatgaaggaagcaaactttgccgcactgaaggtggtcgaaggattcgcaggtaccggggtgttcttgatgagaatctgtggaggagggtgtttaagtccgaatccacccatgaggggagaggggtgaaaatgtccgtccgtgtgtggaatctttgcccagatgggcccctgaaggtacacatctctgtcctgccagaccatgcctggaagaacgccttgtgtgttgacatctgcggtagctgcttgtctgttgcctctctggaggttggtagatacagaaccatactgctccgtagccacgggattggttgtcctgatttcctcttcgtctgtaatcatgaccttttcaatgtccacatttgttttctctgagccttgcttcccaaagatgagaaccccgctctgaggaaaaaacttttcttcatcgtccttgtggcttgccatggccgggcccggattcaccagagagtctctgccattgaggtggtacttggtagctccagtccacgagtattcactgttgttgttatccgcagatgtctttgatactcgctgctggcggtaacagggtccaggaagccagttcctagactggtcccgaatgtcactcgctccggcctgagaaaactgaagccttgactgcgtggtggttccacttggagtgtttgttctgcttaagaaatacaggtactggtcgatgagaggattcatgagacggtccagactctggctgtgagcgtagctgctgtggaaaggaacgtcctcaaaagtgtagctgaaggtaaagttgtttccggtacgcagcatctgagaaggaaagtactccaggcagtaaaatgaagagcgtcctactgcctgactcccgttgttcagggtgaggtatccatactgtggcaccatgaagacgtctgctgggaacggcgggaggcatccttgatgcgccgagccgaggacgtacgggagctggtactccgagtcagtaaacacctgaaccgtgctggtaaggttattggcaatcgtcgtcgtaccgtcattctgcgtgacctctttgacttgaatgttaaagagcttgaagttgagtctcttgggtcggaatccccagttgttgttgatgagtctttgccagtcacgtggtgaaaagtggcagtggaatctgttgaagtcaaaatacccccaaggggtgctgtagccaaagtagtgattgtcgttcgaggctcctgattggctggaaatttgtttgtagaggtggttgttgtaggtgggcagggcccaggttcgggtgctggtggtgatgactctgtcgcccatccatgtggaatcgcaatgccaatttcccgaggaattacccactccgtcggcgccctcgttattgtctgccattggtgcgccactgcctgtagccatcgtattagttcccagaccagagggggctgctggtggctgtccgagaggctgggggtcaggtactgagtctgcgtctccagtctgaccaaaattcaatctttttcttgcaggctgctggcccgcctttccggttcccgaggaggagtctggctccacaggagagtgctctaccggcctcttttttcccggagccgtcttaacaggttcctcaaccaggcccagaggttcaagaaccctctttttcgcctggaagactgctcgtccgaggttgcccccaaaagacgtatcttctttaaggcgctcctgaaactccgcgtcggcgtggttgtacttgaggtacgggttgtctccgctgtcgagctgccggtcgtaggctttgtcgtgctcgagggccgcggcgtctgcctcgttgaccggctctcccttgtcgagtccgttgaagggtccgaggtacttgtacccaggaagcacaagacccctgctgtcgtccttatgccgctctgcgggctttggtggtggtgggccaggtttgagcttccaccactgtcttattccttcagagagagtgtcctcgagccaatctgaaacaataggaagggagtggatgtcagtgtgtgctgcccgggggctctgactacaggtctcccccttcgcgcccgatggtgggacggtatgaataatccggaatatttataggtttttttattacaaaactgttacgaaaacagtaaaatacttatttatttgcgagatggttatcattttaattatctccatgatagatctctatcactgatagggagtacttacctggaagataaccatcggcagccatcttaacaggatccgcgcccgatggtgggacggtatgaataatccggaatatttataggtttttttattacaaaactgttacgaaaacagtaaaatacttatttatttgcgagatggttatcattttaattatctccatgatctattaatattccggagtatacctaggagatccgaaccagataagtgaaatctagttccaaactattttgtcatttttaattttcgtattagcttacgacgctacacccagttcccatctattttgtcactcttccctaaataatccttaaaaactccatttccacccctcccagttcccaactattttgtccgcccacagcggggcatttttcttcctgttatgtttttaatcaaacatcctgccaactccatgtgacaaaccgtcatcttcggctacttt

SEQ ID NO: 23 - protein, 728 aa, synthetic construct
AADGYLPDWLEDNLSEGIREWWDLKPGAPKPKANQQKQDDGRGLVLPGYKYLGPFNGLDKGEPVNAADAAALEHDKAYDQQLKAGDNPYLRYNHADAEFERLQEDTSFGGNLGRAVFQAKKRVLEPLGLVEEGAKTAPGKKRPVEQSPQEPDSSSGIGKTGQQPAKKRLNFGQTGDSESVPDPQPLGEPPATPAAVGTTMASGGGAPMADNNEGADGVGNASGNWHCDSTWLGDRVITTSTRTWALPTYNNHLYKQISSASTGASNDNHYFGYSTPWGYFDFNRFHCHFSPRDWQLINNNWGFRPKRLNFKLFNIQVKEVTTNDGVTTIANNLTSTVQVFSDSEYQLPYVLGSAHQGCLPPFPADVFMIPQYGYLTLNNGSQAVGRSSFYCEYFPSQMLRTGNNFTFSYTFEEVPFHSSYAHSQSLDRLMNPLIDQYLYYLNRTQNQSGSAQNKDLLFSRGSPAGMSVQPKNWLPGPCYRQQRVSKTKTNNNSNFTWTGASKYNLNGRESIINPGTAMASHKDDEDKFFPMSGVMIFGKESAGASNTALDNVMITDEEEIKATNPVATERFGTVAVNFQSSTDPATGDVHAMGALPGMVWQDRDVYLQGPIWAKIPHTDGHFHPSPLMGGFGLKNPPPQILIKNTPVPANPPAEFSATKFASFITQYSTGQVSVEIEWEQKENSKRWNPEVQYTSNYAKSANVDFTVDNNGLYTEPRPIGTRYLTRPL

SEQ ID NO: 24 - protein, 727 aa, synthetic construct
AADGYLPDWLEDTLSEGIRQWWKLKPGPPPPKPAERHKDDSRGLVLPGYKYLGPFNGLDKGEPVNEADAAALEHDKAYDRQLDSGDNPYLKYNHADAEFERLKEDTSFGGNLGRAVFQAKKRVLEPLGLVEEPVKTAPGKKRPVEHSPVEPDSSSGTGKAGQQPARKRLNFGQTGDADSVPDPQPLGQPPAAPSGLGNTMATGSGAPMADNNEGADGVGNSSGNWHCDSTWMGDRVITTSTRTWALPTYNNHLYKQISSQSGASNDNHYFGYSTPWGYFDFNRFHCHFSPRDWQLINNNWGFRPKRLNFKLFNIQVKEVTQNDGTTTIANNLTSTVQVFTDSEYQLPYVLGSAHQGCLPPFPADVFMVPQYGYLTLNNGSQAVGRSSFYCEYFPSQMLRTGNNFTFSYTFEDVPFHSSYAHSQSLDRLMNPLIDQYLYYLSRTNTPSGTTTQSRLQFSQAGASDIRDQSRNWLPGPCYRQQRVSKTSANNNSEYSWTGATKYHLNGRDSLVNPGPAMASHKDDEEKFFPQSGVLIFGKQGSEKTNVDIEKVMITDEEEIRTTNPVATEQYGSVSTNLQRNRQAATADVNTQGVLPGMVWQDRDVYLQGPIWAKIPHTDGHFHPSPLMGGFGLKHPPPQILIKNTPVPANPSTTFSAAKFASFITQYSTGQVSVEIEWEQKENSKRWNPEIQYTSNYNKSVNVDFTVDTNGVYSEPRPIGTRYLTRNL

SEQ ID NO: 25 - protein, 728 aa, synthetic construct
AADGYLPDWLEDNLSEGIREWWALKPGVPQPKANQQHQDNRRGLVLPGYKYLGPGNGLDKGEPVNEADAAALEHDKAYDQQLKAGDNPYLKYNHADAEFERLQEDTSFGGNLGRAVFQAKKRILEPLGLVEEAAKTAPGKKGAVDQSPQEPDSSSGVGKSGKQPARKRLNFGQTGDSESVPDPQPLGEPPAAPTSLGNTMASGGGAPMADNNEGADGVGNSSGNWHCDSQWLGDRVITTSTRTWALPTYNNHLYKQISSQSGASNDNHYFGYSTPWGYFDFNRFHCHFSPRDWQLINNNWGFRPKKLSFKLFNIQVRGVTQNDGTTTIANNLTSTVQVFTDSEYQLPYVLGSAHQGCLPPFPADVFMVPQYGYLTLNNGSQAVGRSSFYCEYFPSQMLRTGNNFQFSYTFEDVPFHSSYAHSQSLDRLMNPLIDQYLYYLNRTQGTTSGTTNQSRLLFSQAGPQSMSLQARNWLPGPCYRQQRLSKTANNNNSNFPWTAASKYHLNGRDSLVNPGPAMASHKDDEEKFFPMHGNLIFGKEGTTASNAELDNVMITDEEEIRTTNPVATEQYGTVANNLQSNTAPTTGTVNHQGALPGMVWQDRDVYLQGPIWAKIPHTDGHFHPSPLMGGFGLKHPPPQIMIKNTPVPANPPTTFSPAKFASFITQYSTGQVSVEIEWEQKENSKRWNPEIQYTSNYNKSVNVDFTVDTNGVYSEPRPIGTRYLTRNL

SEQ ID NO: 26 - protein, 727 aa, synthetic construct
MTDGYLPDWLEDNLSEGVREWWALQPGAPKPKANQQHQDNARGLVLPGYKYLGPGNGLDKGEPVNAADAAALEHDKAYDQQLKAGDNPYLKYNHADAEFQRLQGDTSFGGNLGRAVFQAKKRVLEPLGLVEQAGETAPGKKRPLIESPQQPDSSTGIGKKGKQPAKKKLVFEDETGAGDGPPEGSTSGAMSDDSMRAAAGGAAVEGGQGADGVGNASGDWHCDSTWSEGHVTTTSTRTWVLPTYNNHLYKRLGESLQSNTYNGFSTPWGYFDFNRFHCHFSPRDWQLINNNWGMRPKAMRVKIFNIQVKEVTTSNGETTVANNLTSTVQIFADSSYELPYVMDAGQEGSLPPFPNDVFMVPQYGYCGLVTGNTSQQQTDRNAFYCEYFPSQMLRTGNNFEITYSFEKVPFHSMYAHSQSLDRLMNPLIDQYLWGLQSTTTGTTLNAGTATTNFTKLRPTNFSNFKKNWLPGPSIKQQGFSKTANNYKIPATGSDSLIKYETHSTLDGRWSALTPGPPMATAGPADSKFSNSQLIFAGPKQNGNTATVPGTLIFTSEEELAATNATDTDMWGNLPGGDQSSNLPTVDRLTALGAVPGMVWQNRDIYYQGPIWAKIPHTDGHFHPSPLIGGFGLKHPPPQIFIKNTPVPANPATTFSSTPVNSFITQYSTGQVSVQIDWEQKERSKRWNPEVQFTSNYGQQNSLLWAPDAAGKYTEPRAIGTRYLTHHL

SEQ ID NO: 27 - protein, 716 aa, synthetic construct
SFVDHPPDWLEEVGEGLREFLGLEAGPPKPKPNQQHQDQARGLVLPGYNYLGPGNGLDRGEPVNRADEVAREHDISYNEQLEAGDNPYLKYNHADAEFEKLADDTSFGGNLGKAVFQAKKRVLEPFGLVEEGAKTAPTGKRIDDHFPKRKKARTEEDSKPSTSSDAEAGPSGSQQLQIPAQPASSLGDTMSAGGGGPLGDNNQGADGVGNASGDWHCDSTWMGDRVVTKSTRTWVLPSYNNHQYREIKSGSVDGSNANAYFGYSTPWGYFDFNRFHSHWSPRDWQLINNYWGFRPRSLRVKIFNIQVKEVTVQDSTTTIANNLTSTVQVFTDDDYQLPYVVGNGTEGCLPAFPPQVFTLPQYGYATLNRDNTENPTERSSFFCEYFPSKMLRTGNNFEFTYNFEEVPFHSSFAPSQNLFKLANPLVDQYLYRFVSTNNTGGVQFNKNLAGRYANTYKNWFPGPMGRTQGWNLGSGNRASVSAFATTNRMELEGASYQVPPQPNGMTNNLQGSNTYALENTMIFNSQPANPGTTATYLEGNMLITSESETQPVNRVAYNVGGQMATNNQSTTAPATGTYNLQEIVPGSVWMERDVYLQGPIWAKIPETGAHFHPSPAMGGFGLKHPPPMMLIKNTPVPGNITSFSDVPVSSFITQYSTGQVTVEMEWEKKENSKRWNPEIQYTNNYNDPQFVDFAPDSTGEYRTTRPIGTRYLTRPL

SEQ ID NO: 28 - protein, 728 aa, synthetic construct
AADGYLPDWLEDNLSEGIREWWDLKPGAPKPKANQQKQDDGRGLVLPGYKYLGPFNGLDKGEPVNAADAAALEHDKAYDQQLKAGDNPYLRYNHADAEFERLQEDTSFGGNLGRAVFQAKKRVLEPFGLVEEGAKTAPGKKRPVEQSPQEPDSSSGIGKTGQQPAKKRLNFGQTGDSESVPDPQPLGEPPATPAAVGTTMASGGGAPMADNNEGADGVGNASGNWHCDSTWLGDRVITTSTRTWALPTYNNHLYKQISSASTGASNDNHYFGYSTPWGYFDFNRFHCHFSPRDWQLINNNWGFRPKRLNFKLFNIQVKEVTTNDGVTTIANNLTSTVQVFSDSEYQLPYVLGSAHQGCLPPFPADVFMIPQYGYLTLNNGSQAVGRSSFYCEYFPSQMLRTGNNFTFSYTFEDVPFHSSYAHSQSLDRLMNPLIDQYLYYLNRTQNQSGSAQNKDLLFSRGSPAGMSVQPKNWLPGPCYRQQRVSKTKTNNNSNFTWTGASKYNLNGRESIINPGTAMASHKDDKDKFFPMSGVMIFGKESAGASNTALDNVMITDEEEIKATNPVATERFGTVAVNLQSSTDPATGDVHVMGALPGMVWQDRDVYLQGPIWAKIPHTDGHFHPSPLMGGFGLKHPPPQILIKNTPVPANPPAEFSATKFASFITQYSTGQVSVEIEWEQKENSKRWNPEVQYTSNYAKSANVDFTVDNNGLYTEPRPIGTRYLTRPL

SEQ ID NO: 29 - protein, 729 aa, synthetic construct
AADGYLPDWLEDNLSEGIREWWDLKPGAPKPKANQQKQDNGRGLVLPGYKYLGPFNGLDKGEPVNAADAAALEHDKAYDQQLKAGDNPYLRYNHADAEFERLQEDTSFGGNLGRAVFQAKKRVLEPLGLVEEGAKTAPAKKRPVEPSPQRSPDSSTGIGKKGQQPARKRLNFGQTGDSESVPDPQPLGEPPAAPSSVGGTVAAGGGAPMADNNEGADGVGNASGNWHCDSTWLGDRVITTSTRTWALPTYNNHLYKQISSETAGSTNDNTYFGYSTPWGYFDFNRFHCHFSPRDWQLINNNWGFRPKKLRFKLFNIQVKEVTTNDGVTTIANNLTSTIQVFSDSEYQLPYVLGSAHQGCLPPFPADVFMIPQYGYLTLNNGSQSVGRSSFYCEYFPSQMLRTGNNFEFSYSFEDVPFHSSYAHSQSLDRLMNPLIDQYLYYLARTQSNPGGTAGNRELQFYQGGPSTMAEQAKNWLPGPCFRQQRVSKTLDNNNSNFAWTGATKYHLNGRNSLVNPGVAMATHKDDEDRFFPSSGVLIFGKTGATNKTTLENVLMTNEEEIRPTNPVATEEYGIVSSNLQANTAAQTQVVNNQGALPGMVWQNRDVYLQGPIWAKIPHTDGNFHPSPLMGGFGLKHPPPQILIKNTPVPANPPEVFTPAKFASFITQYSTGQVSVEIEWEQKENSKRWNPEIQYTSNFEKQTGVDFAVDSQGVYSEPRPIGTRYLTRNL

SEQ ID NO: 30 - protein, 730 aa, synthetic construct
AADGYLPDWLEDNLSEGIREWWALKPGAPKPKANQQKQDDGRGLVLPGYKYLGPFNGLDKGEPVNAADAAALEHDKAYDQQLQAGDNPYLRYNHADAEFERLQEDTSFGGNLGRAVFQAKKRVLEPLGLVEEGAKTAPGKKRPVEPSPQRSPDSSTGIGKKGQQPARKRLNFGQTGDSESVPDPQPLGEPPAAPSGVGNTMAAGGGAPMADNNEGADGVGSSSGNWHCDSTWLGDRVITTSTRTWALPTYNNHLYKQISNGTSGGATNDNTYFGYSTPWGYFDFNRFHCHFSPRDWQLINNNWGFRPKRLSFKLFNIQVKEVTQNEGTKTIANNLTSTIQVFTDSEYQLPYVLGSAHQGCLPPFPADVFMIPQYGYLTLNNGSQAVGRSSFYCEYFPSQMLRTGNNFQFTYTFEDVPFHSSYAHSQSLDRLMNPLIDQYLYYLSRTQTTGGTANTQTLGFSQGGPNTMANQAKNWLPGPCYRQQRVSTTTGNNNSNFAWTAGTKYHLNGRNSLANPGIAMATHKDDEERFFPSNGILIFGKQNAARDNADYSDVMLTSEEEIKTTNPVATEEYGIVADNLQQNTAPQIGTVNSQGALPGMVWQNRDVYLQGPIWAKIPHTDGNFHPSPLMGGFGLKHPPPQILIKNTPVPADPPTTFNQSKLNSFITQYSTGQVSVEIEWEQKENSKRWNPEIQYTSNYYKSTSVDFAVNTEGVYSEPRPIGTRYLTRNL

SEQ ID NO: 31 - protein, 728 aa, synthetic construct
AADGYLPDWLEDNLSEGIREWWALKPGAPQPKANQQHQDNARGLVLPGYKYLGPGNGLDKGEPVNAADAAALEHDKAYDQQLKAGDNPYLKYNHADAEFERLKEDTSFGGNLGRAVFQAKKRLLEPLGLVEEAAKTAPGKKRPVEQSPQEPDSSAGIGKSGAQPAKKRLNFGQTGDTESVPDPQPIGEPPAAPSGVGLTMASGGGAPVADNNEGADGVGSSSGNWHCDSQWLGDRVITTSTRTWALPTYNNHLYKQISNSTSGGSSNDNAYFGYSTPWGYFDFNRFHCHFSPRDWQLINNNWGFRPKRLNFKLFNIQVKEVTDNNGVKTIANNLTSTVQVFTDSDYQLPYVLGSAHEGCLPPFPADVFMIPQYGYLTLNDGSQAVGRSSFYCEYFPSQMLRTGNNFQFSYEFENVPFHSSYAHSQSLDRLMNPLIDQYLYYLSKTINGSGQNQQTLKFSVAGPSNMAVQGRNYIPGPSYRQQRVSTTVTNNNSEFAWPGASSWALNGRNSLMNPGPAMASHKEGEDRFFPLSGSLIFGKQGTGRDNVDADKVMITNEEEIKTTNPVATESYGQVATNHQSQAQAQTGWVQNQGILPGMVWQDRDVYLQGPIWAKIPHTDGNFHPSPLMGGFGMKHPPPQILIKNTPVPADPPTAFNKDKLNSFITQYSTGQVSVEIEWEQKENSKRWNPEIQYTSNYYKSNNVEFAVNTEGVYSEPRPIGTRYLTRNL

SEQ ID NO: 32 - protein, 738 aa, synthetic construct
MAADGYLPDWLEDNLSEGIREWWDLKPGAPKPKANQQKQDDGRGLVLPGYKYLGPFNGLDKGEPVNAADAAALEHDKAYDQQLKAGDNPYLRYNHADAEFQERLQEDTSFGGNLGRAVFQAKKRVLEPLGLVEEGAKTAPGKKRPVEPSPQRSPDSSTGIGKKGQQPAKKRLNFGQTGDSESVPDPQPIGEPPAGPSGLGSGTMAAGGGAPMADNNEGADGVGSSSGNWHCDSTWLGDRVITTSTRTWALPTYNNHLYKQISNGTSGGSTNDNTYFGYSTPWGYFDFNRFHCHFSPRDWQRLINNNWGFRPKRLNFKLFNIQVKEVTQNEGTKTIANNLTSTIQVFTDSEYQLPYVLGSAHQGCLPPFPADVFMIPQYGYLTLNNGSQAVGRSSFYCLEYFPSQMLRTGNNFEFSYQFEDVPFHSSYAHSQSLDRLMNPLIDQYLYYLSRTQSTGGTAGTQQLLFSQAGPNNMSAQAKNWLPGPCYRQQRVSTTLSQNNNSNFAWTGATKYHLNGRDSLVNPGVAMATHKDDEERFFPSSGVLMFGKQGAGKDNVDYSSVMLTSEEEIKTTNPVATEQYGVVADNLQQQNAAPIVGAVNSQGALPGMVWQNRDVYLQGPIWAKIPHTDGNFHPSPLMGGFGLKHPPPQILIKNTPVPADPPTTFSQAKLASFITQYSTGQVSVEIEWELQKENSKRWNPEIQYTSNYYKSTNVDFAVNTDGTYSEPRPIGTRYLTRNL

SEQ ID NO: 33 - protein, 733 aa, synthetic construct
MAADGYLPDWLEDNLSEGIREWWDLKPGAPKPKANQQKQDDGRGLVLPGYKYLGPFNGLDKGEPVNAADAAALEHDKAYDQQLKAGDNPYLRYNHADAEFQERLQEDTSFGGNLGRAVFQAKKRVLEPLGLVEEGAKTAPGKKRPLESPQEPDSSSGIGKKGKQPARKRLNFEEDTGAGDGPPEGSDTSAMSSDIEMRAAPGGNAVDAGQGSDGVGNASGDWHCDSTWSEGKVTTTSTRTWVLPTYNNHLYLRLGTTSSSNTYNGFSTPWGYFDFNRFHCHFSPRDWQRLINNNWGLRPKAMRVKIFNIQVKEVTTSNGETTVANNLTSTVQIFADSSYELPYVMDAGQEGSLPPFPNDVFMVPQYGYCGIVTGENQNQTDRNAFYCLEYFPSQMLRTGNNFEMAYNFEKVPFHSMYAHSQSLDRLMNPLLDQYLWHLQSTTSGETLNQGNAATTFGKIRSGDFAFYRKNWLPGPCVKQQRFSKTASQNYKIPASGGNALLKYDTHYTLNNRWSNIAPGPPMATAGPSDGDFSNAQLIFPGPSVTGNTTTSANNLLFTSEEEIAATNPRDTDMFGQIADNNQNATTAPITGNVTAMGVLPGMVWQNRDIYYQGPIWAKIPHADGHFHPSPLIGGFGLKHPPPQIFIKNTPVPANPATTFTAARVDSFITQYSTGQVAVQIEWEIEKERSKRWNPEVQFTSNYGNQSSMLWAPDTTGKYTEPRVIGSRYLTNHL

SEQ ID NO: 34 - protein, 741 aa, synthetic construct
MAADGYLPDWLEDNLSEGIREWWALKPGAPQPKANQQHQDNGRGLVLPGYKYLGPFNGLDKGEPVNEADAAALEHDKAYDKQLEQGDNPYLKYNHADAEFQQRLATDTSFGGNLGRAVFQAKKRILEPLGLVEEGVKTAPGKKRPLEKTPNRPTNPDSGKAPAKKKQKDGEPADSARRTLDFEDSGAGDGPPEGSSSGEMSHDAEMRAAPGGNAVEAGQGADGVGNASGDWHCDSTWSEGRVTTTSTRTWVLPTYNNHLYLRIGTTANSNTYNGFSTPWGYFDFNRFHCHFSPRDWQRLINNNWGLRPKSMRVKIFNIQVKEVTTSNGETTVANNLTSTVQIFADSTYELPYVMDAGQEGSFPPFPNDVFMVPQYGYCGVVTGKNQNQTDRNAFYCLEYFPSQMLRTGNNFEVSYQFEKVPFHSMYAHSQSLDRMMNPLLDQYLWHLQSTTTGNSLNQGTATTTYGKITTGDFAYYRKNWLPGACIKQQKFSKNANQNYKIPASGGDALLKYDTHTTLNGRWSNMAPGPPMATAGAGDSDFSNSQLIFAGPNPSGNTTTSSNNLLFTSEEEIATTNPRDTDMFGQIADNNQNATTAPHIANLDAMGIVPGMVWQNRDIYYQGPIWAKVPHTDGHFHPSPLMGGFGLKHPPPQIFIKNTPVPANPNTTFSAARINSFLTQYSTGQVAVQIDWEIQKEHSKRWNPEVQFTSNYGTQNSMLWAPDNAGNYHELRAIGSRFLTHH